European Patent Application EP 4 450 092 A1, published October 23, 2024. Title: MODIFIED OLIGONUCLEOTIDE-DRUG CONJUGATE AND USE THEREOF. Applicant: INTEROLIGO Corporation. Application KR PCT/KR2022/017440, filed November 8, 2022. The sequence listing filed with the application follows.

SEQUENCE LISTING (33 sequences)

SEQ ID NO: 1 - DNA, 26 bp, synthetic construct
  source 1..26: mol_type = other DNA
ggtggtggtggttgtggtggtggtgg

SEQ ID NO: 2 - DNA, 26 bp, synthetic construct
  source 1..26: mol_type = other DNA
  modified_base 15: mod_base = OTHER; note = deoxyuridine(dU)
ggtggtggtggttgnggtggtggtgg

SEQ ID NO: 3 - DNA, 26 bp, synthetic construct
  source 1..26: mol_type = other DNA
  modified_base 13: mod_base = OTHER; note = deoxyuridine(dU)
ggtggtggtggtngtggtggtggtgg

SEQ ID NO: 4 - DNA, 26 bp, synthetic construct
  source 1..26: mol_type = other DNA
  modified_base 12: mod_base = OTHER; note = deoxyuridine(dU)
  modified_base 13: mod_base = OTHER; note = Gemcitabine
ggtggtggtggnngtggtggtggtgg

SEQ ID NO: 5 - DNA, 26 bp, synthetic construct
  source 1..26: mol_type = other DNA
  modified_base 12: mod_base = OTHER; note = deoxyuridine(dU)
  modified_base 14: mod_base = OTHER; note = gemcitabine
ggtggtggtggntntggtggtggtgg

SEQ ID NO: 6 - DNA, 26 bp, synthetic construct
  source 1..26: mol_type = other DNA
  modified_base 13: mod_base = OTHER; note = deoxyuridine(dU)
  modified_base 14: mod_base = OTHER; note = gemcitabine
ggtggtggtggtnntggtggtggtgg

SEQ ID NO: 7 - DNA, 26 bp, synthetic construct
  source 1..26: mol_type = other DNA
  modified_base 13: mod_base = OTHER; note = deoxyuridine(dU)
  modified_base 15: mod_base = OTHER; note = gemcitabine
ggtggtggtggtngnggtggtggtgg

SEQ ID NO: 8 - DNA, 26 bp, synthetic construct
  source 1..26: mol_type = other DNA
  modified_base 13: mod_base = OTHER; note = deoxyuridine(dU)
  modified_base 12: mod_base = OTHER; note = gemcitabine
  modified_base 15: mod_base = OTHER; note = gemcitabine
ggtggtggtggnngnggtggtggtgg

SEQ ID NO: 9 - DNA, 26 bp, synthetic construct
  source 1..26: mol_type = other DNA
  modified_base 13: mod_base = OTHER; note = deoxyuridine(dU)
  modified_base 24: mod_base = OTHER; note = gemcitabine
ggtggtggtggtngtggtggtggngg

SEQ ID NO: 10 - DNA, 26 bp, synthetic construct
  source 1..26: mol_type = other DNA
  modified_base 15: mod_base = OTHER; note = deoxyuridine(dU)
  modified_base 24: mod_base = OTHER; note = gemcitabine
ggtggtggtggttgnggtggtggngg

SEQ ID NO: 11 - DNA, 28 bp, synthetic construct
  source 1..28: mol_type = other DNA
  modified_base 27: mod_base = OTHER; note = gemcitabine
  modified_base 28: mod_base = OTHER; note = gemcitabine
ggtggtggtggttgtggtggtggtggnn

SEQ ID NO: 12 - DNA, 28 bp, synthetic construct
  source 1..28: mol_type = other DNA
  modified_base 27: mod_base = OTHER; note = 5-fluorodeoxyuridine
  modified_base 28: mod_base = OTHER; note = 5-fluorodeoxyuridine(5-FdU)
ggtggtggtggttgtggtggtggtggnn

SEQ ID NO: 13 - DNA, 26 bp, synthetic construct
  source 1..26: mol_type = other DNA
  modified_base 15: mod_base = OTHER; note = deoxyuridine(dU)-acrylamide-C6-NH2
ggtggtggtggttgnggtggtggtgg

SEQ ID NO: 14 - DNA, 26 bp, synthetic construct
  source 1..26: mol_type = other DNA
  modified_base 13: mod_base = OTHER; note = deoxyuridine(dU)-acrylamide-C6-NH2
ggtggtggtggtngtggtggtggtgg

SEQ ID NO: 15 - DNA, 26 bp, synthetic construct
  source 1..26: mol_type = other DNA
  modified_base 12: mod_base = OTHER; note = deoxyuridine(dU)-acrylamide-C6-NH2
  modified_base 13: mod_base = OTHER; note = gemcitabine
ggtggtggtggnngtggtggtggtgg

SEQ ID NO: 16 - DNA, 32 bp, synthetic construct
  source 1..32: mol_type = other DNA
  modified_base 1: mod_base = OTHER; note = gemcitabine
  modified_base 2: mod_base = OTHER; note = gemcitabine
nntggtggtggtggttgtggtggtggtggtgg

SEQ ID NO: 17 - DNA, 26 bp, synthetic construct
  source 1..26: mol_type = other DNA
  modified_base 12: mod_base = OTHER; note = deoxyuridine(dU)-acrylamide-C6-NH2
  modified_base 14: mod_base = OTHER; note = gemcitabine
ggtggtggtggntntggtggtggtgg

SEQ ID NO: 18 - DNA, 26 bp, synthetic construct
  source 1..26: mol_type = other DNA
  modified_base 13: mod_base = OTHER; note = deoxyuridine(dU)-acrylamide-C6-NH2
  modified_base 14: mod_base = OTHER; note = gemcitabine
ggtggtggtggtnntggtggtggtgg

SEQ ID NO: 19 - DNA, 26 bp, synthetic construct
  source 1..26: mol_type = other DNA
  modified_base 13: mod_base = OTHER; note = deoxyuridine(dU)-acrylamide-C6-NH2
  modified_base 15: mod_base = OTHER; note = gemcitabine
ggtggtggtggtngnggtggtggtgg

SEQ ID NO: 20 - DNA, 26 bp, synthetic construct
  source 1..26: mol_type = other DNA
  modified_base 13: mod_base = OTHER; note = deoxyuridine(dU)-acrylamide-C6-NH2
  modified_base 12: mod_base = OTHER; note = gemcitabine
  modified_base 15: mod_base = OTHER; note = gemcitabine
ggtggtggtggnngnggtggtggtgg

SEQ ID NO: 21 - DNA, 26 bp, synthetic construct
  source 1..26: mol_type = other DNA
  modified_base 13: mod_base = OTHER; note = deoxyuridine(dU)-acrylamide-C6-NH2
  modified_base 24: mod_base = OTHER; note = gemcitabine
ggtggtggtggtngtggtggtggngg

SEQ ID NO: 22 - DNA, 26 bp, synthetic construct
  source 1..26: mol_type = other DNA
  modified_base 15: mod_base = OTHER; note = deoxyuridine(dU)-acrylamide-C6-NH2
  modified_base 24: mod_base = OTHER; note = gemcitabine
ggtggtggtggttgnggtggtggngg

SEQ ID NO: 23 - DNA, 28 bp, synthetic construct
  source 1..28: mol_type = other DNA
  modified_base 27: mod_base = OTHER; note = gemcitabine
  modified_base 28: mod_base = OTHER; note = gemcitabine
  modified_base 1: mod_base = OTHER; note = deoxyguanosine(dG)-C6-NH2
ggtggtggtggttgtggtggtggtggnn

SEQ ID NO: 24 - DNA, 26 bp, synthetic construct
  source 1..26: mol_type = other DNA
  modified_base 1: mod_base = OTHER; note = deoxyguanosine(dG)-C6-SS-C6-OH
ggtggtggtggttgtggtggtggtgg

SEQ ID NO: 25 - DNA, 26 bp, synthetic construct
  source 1..26: mol_type = other DNA
  modified_base 1: mod_base = OTHER; note = deoxyguanosine(dG)-C6-SH
ggtggtggtggttgtggtggtggtgg

SEQ ID NO: 26 - DNA, 28 bp, synthetic construct
  source 1..28: mol_type = other DNA
  modified_base 27: mod_base = OTHER; note = gemcitabine
  modified_base 28: mod_base = OTHER; note = gemcitabine
  variation 1: note = deoxyguanosine(dG)-C6-SS-C6-OH
ggtggtggtggttgtggtggtggtggnn

SEQ ID NO: 27 - DNA, 28 bp, synthetic construct
  source 1..28: mol_type = other DNA
  modified_base 27: mod_base = OTHER; note = gemcitabine
  modified_base 28: mod_base = OTHER; note = gemcitabine
  variation 1: note = deoxyguanosine(dG)-C6-SH
ggtggtggtggttgtggtggtggtggnn

SEQ ID NO: 28 - DNA, 26 bp, synthetic construct
  source 1..26: mol_type = other DNA
  modified_base 1: mod_base = OTHER; note = deoxyguanosine(dG)-C6-NH2
ggtggtggtggttgtggtggtggtgg

SEQ ID NO: 29 - DNA, 28 bp, synthetic construct
  source 1..28: mol_type = other DNA
  modified_base 27: mod_base = OTHER; note = gemcitabine
  modified_base 28: mod_base = OTHER; note = gemcitabine
  variation 1: note = deoxyguanosine(dG)-C6-NH2
ggtggtggtggttgtggtggtggtggnn

SEQ ID NO: 30 - DNA, 26 bp, synthetic construct
  source 1..26: mol_type = other DNA
  modified_base 13: mod_base = OTHER; note = deoxyuridine(dU)-acrylamide-C6-NH2
ggtggtggtggtngtggtggtggtgg

SEQ ID NO: 31 - DNA, 26 bp, synthetic construct
  source 1..26: mol_type = other DNA
  modified_base 12: mod_base = OTHER; note = gemcitabine
  modified_base 15: mod_base = OTHER; note = gemcitabine
  variation 13: note = deoxyuridine(dU)-acrylamide-C6-NH2
ggtggtggtggnngnggtggtggtgg

SEQ ID NO: 32 - DNA, 26 bp, synthetic construct
  source 1..26: mol_type = other DNA
  modified_base 1: mod_base = OTHER; note = deoxyguanosine(dG)-C6-NH2
ggtggtggtggttgtggtggtggtgg

SEQ ID NO: 33 - DNA, 28 bp, synthetic construct
  source 1..28: mol_type = other DNA
  modified_base 27: mod_base = OTHER; note = gemcitabine
  modified_base 28: mod_base = OTHER; note = gemcitabine
  modified_base 1: mod_base = OTHER; note = deoxyguanosine(dG)-C6-NH2
ggtggtggtggttgtggtggtggtggnn